European Patent Specification EP 3 674 423 B1, published September 2, 2026. Title: COMPOSITIONS AND ASSAYS TO DETECT SWINE H1N1 INFLUENZA A VIRUS, SEASONAL H1 INFLUENZA A VIRUS, AND SEASONAL H3 INFLUENZA A VIRUS NUCLEIC ACIDS. Applicant: Gen-Probe Incorporated TYLER, Ejan. The sequence listing filed with the application follows.

SEQUENCE LISTING (106 sequences)

SEQ ID NO: 1 - DNA, 19 bp, Influenza A virus
aagtcgaaacccaggaaac

SEQ ID NO: 2 - DNA, 18 bp, Influenza A virus
catgcccacttgctactg

SEQ ID NO: 3 - DNA, 22 bp, Influenza A virus
catacacacaagcaggcaggca

SEQ ID NO: 4 - DNA, 24 bp, Influenza A virus
aagacctcattttcctggcacggt

SEQ ID NO: 5 - DNA, 18 bp, Influenza A virus
cacggtcagcactcattc

SEQ ID NO: 6 - DNA, 20 bp, Influenza A virus
ttcaaagtcatgcccacttg

SEQ ID NO: 7 - DNA, 25 bp, Influenza A virus
atcagttgcacataaatcctgcctg

SEQ ID NO: 8 - DNA, 20 bp, Influenza A virus
attggtggaatcgggagatt

SEQ ID NO: 9 - DNA, 23 bp, Influenza A virus
aggtatttatttcttctctcatc

SEQ ID NO: 10 - DNA, 26 bp, Influenza A virus
tccaaatgtgcactgaactcaaactc

SEQ ID NO: 11 - DNA, 27 bp, Influenza A virus
tagtcgtccatcataatcactgagttt

SEQ ID NO: 12 - DNA, 17 bp, Influenza A virus
tggcgtctcaaggcacc

SEQ ID NO: 13 - DNA, 21 bp, Influenza A virus
ttccaccaatcattcttccga

SEQ ID NO: 14 - DNA, 27 bp, Influenza A virus
atcatatgaacaaatggagactggtgg

SEQ ID NO: 15 - DNA, 24 bp, Influenza A virus
cgccaggatgccacagaaatcaga

SEQ ID NO: 16 - DNA, 25 bp, Influenza A virus
tgctctgatttctgtggcatcctgg

SEQ ID NO: 17 - DNA, 19 bp, Influenza A virus
tagaagagcatcccagtgc

SEQ ID NO: 18 - DNA, 18 bp, Influenza A virus
ccattgtttgcttggcgc

SEQ ID NO: 19 - DNA, 26 bp, Influenza A virus
aaggaccctaagaaaacaggaggacc

SEQ ID NO: 20 - DNA, 29 bp, Influenza A virus
ttcttctttgtcataaaggatgagttctc

SEQ ID NO: 21 - DNA, 20 bp, Influenza A virus
caacctgaatgatgccacat

SEQ ID NO: 22 - DNA, 20 bp, Influenza A virus
tcggtcattgattccacgtt

SEQ ID NO: 23 - DNA, 23 bp, Influenza A virus
agagcgcttgttcgcaccggaat

SEQ ID NO: 24 - DNA, 27 bp, Influenza A virus
cagaatgtgctctctaatgcaaggttc

SEQ ID NO: 25 - DNA, 31 bp, Influenza A virus
tcattctgattaactccattgctattgttcc

SEQ ID NO: 26 - DNA, 19 bp, Influenza A virus
agtggtcagcctgatgaga

SEQ ID NO: 27 - DNA, 22 bp, Influenza A virus
cttaaatcttcaaatgcagcag

SEQ ID NO: 28 - DNA, 27 bp, Influenza A virus
caaatgaaaacccagctcacaagagtc

SEQ ID NO: 29 - DNA, 24 bp, Influenza A virus
tggcatgccatccacaccaattga

SEQ ID NO: 30 - DNA, 18 bp, Influenza A virus
actgggccataaggacca

SEQ ID NO: 31 - DNA, 18 bp, Influenza A virus
ccgctgaatgctgccata

SEQ ID NO: 32 - DNA, 29 bp, Influenza A virus
agtggaggaaataccaatcaacaaaaggc

SEQ ID NO: 33 - DNA, 23 bp, Influenza A virus
cgctgcactgagaatgtaggctg

SEQ ID NO: 34 - DNA, 20 bp, Influenza A virus
gcgaacaattcaacagacac

SEQ ID NO: 35 - DNA, 18 bp, Influenza A virus
gatttcccaggatccagc

SEQ ID NO: 36 - DNA, 30 bp, Influenza A virus
tagacacagtactagaaaagaatgtaacag

SEQ ID NO: 37 - DNA, 23 bp, Influenza A virus
atgcaatggggctacccctctta

SEQ ID NO: 38 - DNA, 20 bp, Influenza A virus
acgtgttacccaggagattt

SEQ ID NO: 39 - DNA, 20 bp, Influenza A virus
cttggggaatatctcaaacc

SEQ ID NO: 40 - DNA, 27 bp, Influenza A virus
tcgattatgaggagctaagagagcaat

SEQ ID NO: 41 - DNA, 27 bp, Influenza A virus
attgctctcttagctcctcataatcga

SEQ ID NO: 42 - DNA, 18 bp, Influenza A virus
gtaacggcagcatgtcct

SEQ ID NO: 43 - DNA, 20 bp, Influenza A virus
tagagactttgttggtcagc

SEQ ID NO: 44 - DNA, 23 bp, Influenza A virus
tggtgaatgccccatagcacgag

SEQ ID NO: 45 - DNA, 22 bp, Influenza A virus
agaatgaactattactggacac

SEQ ID NO: 46 - DNA, 20 bp, Influenza A virus
ggactggtgtatctgaaatg

SEQ ID NO: 47 - DNA, 26 bp, Influenza A virus
tagagccgggagacaaaataacattc

SEQ ID NO: 48 - DNA, 26 bp, Influenza A virus
actggaaatctagtggtaccgagata

SEQ ID NO: 49 - DNA, 27 bp, Influenza A virus
taccagatccagcatttctttccattg

SEQ ID NO: 50 - DNA, 20 bp, Influenza A virus
agcacaaaattgagactggc

SEQ ID NO: 51 - DNA, 19 bp, Influenza A virus
cctgctcattttgatggtg

SEQ ID NO: 52 - DNA, 24 bp, Influenza A virus
caggattgaggaatgtcccgtcta

SEQ ID NO: 53 - DNA, 23 bp, Influenza A virus
accgtaccatccatctaccatcc

SEQ ID NO: 54 - DNA, 20 bp, Influenza A virus
acagttcacagcagtaggta

SEQ ID NO: 55 - DNA, 22 bp, Influenza A virus
ctggcttcttaccttttcatat

SEQ ID NO: 56 - DNA, 27 bp, Influenza A virus
ttgatgatggtttcctggacatttgga

SEQ ID NO: 57 - DNA, 29 bp, Influenza A virus
tcttcacatttgaatcgtggtagtccaaa

SEQ ID NO: 58 - DNA, 28 bp, Influenza A virus
tcattttccaatagaaccaacagttcgg

SEQ ID NO: 59 - DNA, 24 bp, Influenza A virus
gaagcaaaattaaacagagaagaa

SEQ ID NO: 60 - DNA, 21 bp, Influenza A virus
tagagcacatccagaaactga

SEQ ID NO: 61 - DNA, 29 bp, Influenza A virus
atcaacaaggatttaccagattttggcga

SEQ ID NO: 62 - DNA, 28 bp, Influenza A virus
accaatgaactggcgacagttgaataga

SEQ ID NO: 63 - DNA, 20 bp, Influenza A virus
aggtttgtttggagccattg

SEQ ID NO: 64 - DNA, 20 bp, Influenza A virus
ttgttgaattctttgcccac

SEQ ID NO: 65 - DNA, 24 bp, Influenza A virus
tcattgaaggggggtggactggaa

SEQ ID NO: 66 - DNA, 25 bp, Influenza A virus
tggactggaatggtagatggttggt

SEQ ID NO: 67 - DNA, 33 bp, Influenza A virus
tcattttctcaattacagaattcaccttgtttg

SEQ ID NO: 68 - DNA, 22 bp, Influenza A virus
atcatacagaaaatgcttatgt

SEQ ID NO: 69 - DNA, 18 bp, Influenza A virus
magcagagtccagtagta

SEQ ID NO: 70 - DNA, 29 bp, Influenza A virus
ttcacattatagcagaagattcaccccag

SEQ ID NO: 71 - DNA, 24 bp, Influenza A virus
accccagaaatagccaaaagaccc

SEQ ID NO: 72 - DNA, 23 bp, Influenza A virus
ttgaggcaaatggaaatctaata

SEQ ID NO: 73 - DNA, 21 bp, Influenza A virus
tacattctggaaaggaagact

SEQ ID NO: 74 - DNA, 27 bp, Influenza A virus
agtagaggctttggatcaggaatcatc

SEQ ID NO: 75 - DNA, 28 bp, Influenza A virus
tgtttatagctccctgaggtgtttgaca

SEQ ID NO: 76 - DNA, 28 bp, Influenza A virus
cattggtgcatttgaggtgatgattcct

SEQ ID NO: 77 - DNA, 20 bp, Influenza A virus
actaatgctactgagctggt

SEQ ID NO: 78 - DNA, 21 bp, Influenza A virus
cttattttggaagccatcaca

SEQ ID NO: 79 - DNA, 27 bp, Influenza A virus
atccttgatggagaaaactgcacacta

SEQ ID NO: 80 - DNA, 27 bp, Influenza A virus
agggtctcccaatagagcatctattag

SEQ ID NO: 81 - DNA, 27 bp, Influenza A virus
tagtgtgcagttttctccatcaaggat

SEQ ID NO: 82 - DNA, 22 bp, Influenza A virus
aagactatcattgctttgagct

SEQ ID NO: 83 - DNA, 20 bp, Influenza A virus
tgaaccagctcagtagcatt

SEQ ID NO: 84 - DNA, 31 bp, Influenza A virus
cttcaatttggtcattcgtgattgttttcac

SEQ ID NO: 85 - DNA, 19 bp, Influenza A virus
ctctattgggagaccctca

SEQ ID NO: 86 - DNA, 22 bp, Influenza A virus
ctttcattgttaaactccagtg

SEQ ID NO: 87 - DNA, 29 bp, Influenza A virus
tgtgatggcttccaaaataagaaatggga

SEQ ID NO: 88 - DNA, 21 bp, Influenza A virus
tgctcaagcatcaggaagaat

SEQ ID NO: 89 - DNA, 20 bp, Influenza A virus
ccctaggagcaattagattc

SEQ ID NO: 90 - DNA, 29 bp, Influenza A virus
tctaccaaaagaagccaacaaactgtaat

SEQ ID NO: 91 - DNA, 27 bp, Influenza A virus
tgctgttaatcaaaagtatgtctcccg

SEQ ID NO: 92 - DNA, 22 bp, Influenza A virus
agctcaataatgagatcagatg

SEQ ID NO: 93 - DNA, 20 bp, Influenza A virus
ttccctcccaaccattttct

SEQ ID NO: 94 - DNA, 28 bp, Influenza A virus
ccaaatggaagcattcccaatgacaaac

SEQ ID NO: 95 - DNA, 28 bp, Influenza A virus
caaatatgcctctagtttgtttctctgg

SEQ ID NO: 96 - DNA, 20 bp, Influenza A virus
tctcaaaagcactcaagcag

SEQ ID NO: 97 - DNA, 18 bp, Influenza A virus
ctccgcgttgtatgacca

SEQ ID NO: 98 - DNA, 27 bp, Influenza A virus
caaatcaatgggaagctgaatagrttg

SEQ ID NO: 99 - DNA, 20 bp, Influenza A virus
cctggagaaccaacatacaa

SEQ ID NO: 100 - DNA, 20 bp, Influenza A virus
caggcattgtcacatttgtg

SEQ ID NO: 101 - DNA, 30 bp, Influenza A virus
tgatctaactgactcagaaatgaacaaact

SEQ ID NO: 102 - DNA, 26 bp, Influenza A virus
atcctcagcattttccctcagttgct

SEQ ID NO: 103 - DNA, 1701 bp, Influenza A virus
atgaaggcaatactagtagttctgctatatacatttgcaaccgcaaatgcagacacattatgtataggttatcatgcgaacaattcaacagacactgtagacacagtactagaaaagaatgtaacagtaacacactctgttaaccttctagaatacaagcataacgggaaactatgcaaactaagaggggtagccccattgcatttgggtaaatgtaacattgctggctggatcctgggaaatccagagtgtgaatcactctccacagcaagctcatggtcctacattgtggaaacatctagttcagacaatggaacgtgttacccaggagatttcatcgattatgaggagctaagagagcaattgagctcagtgtcatcatttgaaaggtttgagatattccccaagacaagttcatggcccaatcatgactcgaacaaaggtgtaacggcagcatgtcctcatgctggagcaaaaagcttctacaaaaatttaatatggctagttaaaaaagaaaattcatacccaaagctcagcaaatcctacattaatgataaagggaaagaagtcctcgtgctatggggcattcaccatccatctactagtgctgaccaacaaagtctctatcagaatgcagatgcatatgtttttgtggggacatcaagatacagcaagaagttcaagccggaaatagcaataagacccaaagtgagggatcaagaagggagaatgaactattactggacactagtagagccgggagacaaaataacattcgaagcaactggaaatctagtggtaccgagatatgcattcgcaatggaaagaaatgctggatctggtattatcatttcagatacaccagtccacgattgcaatacaacttgtcagacacccaagggtgctataaacaccagcctcccatttcagaatatacatccgatcacaattggagaatgtccaaaatatgtaaaaagcacaaaattgagactggccacaggattgaggaatgtcccgtctattcaatctagaggcctatttggggccattgccggtttcattgaaggggggtggacagggatggtagatggatggtacggttatcaccatcaaaatgagcaggggtctggatatgcagccgacctgaagagcacacagaatgccattgacgagattactaacaaagtaaattctgttattgaaaagatgaatacacagttcacagcagtaggtaaagagttcaaccacctggaaaaaagaatagagaatttaaataaaaaggttgatgatggtttcctggacatttggacttacaattccgaactgttggttctattggaaaatgaaagaactttggactaccacgattcaaatgtgaagaacttatatgaaaaggtaagaagccagttaaaaaacaatgccaaggaaattggaaacggctgctttgaattttaccacaaatgcgataacacgtgcatggaaagtgtcaaaaatgggacttatgactacccaaaatactcagaggaagcaaaattaaacagagaagaaatagatggggtaaagctggaatcaacaaggatttaccagattttggcgatctattcaactgtcgccagttcattggtactggtagtctccctgggggcaatcagtttctggatgtgctctaatgggtctctacagtgtagaatatgtatttaa

SEQ ID NO: 104 - DNA, 1577 bp, Influenza A virus
agggtagataatcactcactgagtgacatcgaagccatggcgtctcaaggcaccaaacgatcatatgaacaaatggagactggtggggagcgccaggatgccacagaaatcagagcatctgtcggaagaatgattggtggaatcgggagattctacatccaaatgtgcactgaactcaaactcagtgattatgatggacgactaatccagaatagcataacaatagagaggatggtgctttctgcttttgatgagagaagaaataaatatctagaagagcatcccagtgctgggaaggaccctaagaaaacaggaggacccatatatagaagaatagacggaaagtggatgagagaactcatcctttatgacaaagaagaaataaggagagtttggcgccaagcaaacaatggcgaagatgcaacagcaggtcttactcatatcatgatttggcattccaacctgaatgatgccacatatcagagaacaagagcgcttgttcgcaccggaatggatcccagaatgtgctctctaatgcaaggttcaacacttcccagaaggtctggtgccgcaggtgctgcggtgaaaggagttggaacaatagcaatggagttaatcagaatgatcaaacgtggaatcaatgaccgaaatttctggaggggtgaaaatggacgaaggacaagggttgcttatgaaagaatgtgcaatatcctcaaaggaaaatttcaaacagctgcccagagggcaatgatggatcaagtaagagaaagtcgaaacccaggaaacgctgagattgaagacctcattttcctggcacggtcagcactcatcctaaggggatcagttgcacataaatcctgcctgcctgcttgtgtgtatgggcttgcagtagcaagtgggcatgactttgaaagggaagggtactcactggtcgggatagacccattcaaattactccaaaacagccaagtggtcagcctgatgagaccaaatgaaaacccagctcacaagagtcaattggtgtggatggcatgccactctgctgcatttgaagatttaagagtatcaagtttcataagaggaaagaaagtgattccaagaggaaagctttccacaagaggggtccagattgcttcaaatgagaatgtggaaaccatggactccaataccctggaactaagaagcagatactgggccataaggaccaggagtggaggaaataccaatcaacaaaaggcatccgcaggccagatcagtgtgcagcctacattctcagtgcagcggaatctcccttttgaaagagcaactgttatggcagcattcagcgggaacaatgaaggacggacatccgacatgcgaacagaagttataagaatgatggaaagtgcaaagccagaagatttgtccttccaggggcggggagtcttcgagctctcggacgaaaaggcaacgaacccgatcgtgccttcctttgacatgagtaatgaagggtcttatttcttcggagacaatgcagaggagtatgacagttgaggaaaaatacccttgtttctactggtcatagctgttttcctgaa

SEQ ID NO: 105 - DNA, 1066 bp, Influenza A virus
gacacaatatgtataggctaccatgccaacaactcgaccgacactgttgacacagtacttgagaagaatgtgacagtgacacactctgtcaacctacttgaggacagtcacaatggaaaactatgtctactaaaaggaatagccccactacaattgggtaattgcagcgttgccggatggatcctaggaaacccagaatgcgaattactgatttccaaggaatcatggtcctacattgtagagacaccaaatcctgagaatggaacatgttacccagggtatttcgccgactatgaggagctgagagagcaattgagttcagtatcttcatttgagaggttcgaaatattccccaaagagagctcatggcccaaccacaccgtaaccggagtatcagcatcatgctcccataacgggaaaagcagtttttacagaaatttgctatggctgacggggaagaatggtttgtatccaaacctgagcaagtcctatgcaaacaacaaagagaaagaagtccttgtactgtggggtgttcatcacccgcctaacatagggaaccaaagggccctctatcatacagaaaatgcttatgtctctgtagtgtcttcacattatagcagaagattcaccccagaaatagccaaaagacccaaggtgagagatcaggaaggaagaatcaactactactggactctgcttgaacccggggatacaataatatttgaggcaaatggaaatctaatagcgccaaggtttgctttcgcactgagtagaggctttggatcaggaatcatcacctcaaatgcaccaatggatgaatgtgatgcgaaatgtcaaacacctcagggagctataaacagcagtcttcctttccagaatgtacacccagtcacaataggagagtgtccaaagtatgtcaggagtgcaaaattaagaatggttacaggactaaggaacatcccatccattcaatccagaggtttgtttggagccattgccggtttcattgaaggggggtggactggaatggtagatggttggtatggttatcaccatcagaatgagc

SEQ ID NO: 106 - DNA, 1701 bp, Influenza A virus
atgaagactatcattgctttgagctacattttatgtctggttttcactcaaaaacttcccggaaatgacaacagcacggcaacgctgtgcctggggcaccatgcagtgccaaacggaacgctagtgaaaacaatcacgaatgaccaaattgaagtgactaatgctactgagctggttcagagttcctcaacaggtagaatatgcgacagtcctcaccaaatccttgatggagaaaactgcacactaatagatgctctattgggagaccctcattgtgatggcttccaaaataaggaatgggacctttttgttgaacgcagcaaagcctacagcaactgttacccttatgatgtgccggattatgtctcccttaggtcactagttgcctcatcaggcacgctggagtttaacaatgaaagcttcaattggactggagtcgctcagaatggaacaagctctgcttgcaaaaggagatctgataaaagtttctttagtagattgaattggttgcaccaattaaaatacaaatatccagcactgaacgtgactatgccaaacaatgaaaaatttgacaaattgtacatttggggggttcaccacccgggtacagacagtgaccaaatcagcctatatgctcaagcatcagggagagtcacagtctctaccaaaagaagccaacaaactgtaatcccgaatatcggatctagaccctgggtaaggggtgtctccagcagaataagcatctattggacaatagtaaaaccgggagacatacttttgattaacagcacagggaatctaattgctcctcggggttatttcaaaatacgaagtgggaaaagctcaataatgaggtcagatgcacccattggcaaatgcaattctgaatgcatcactccaaatggaagcattcccaatgacaaaccatttcaaaatgtaaacaggatcacatatgggccctgtcccagatatgttaagcaaaacactctgaaattggcaacagggatgcggaatgtgccagagaaacaaactagaggcatattcggtgcaatcgcgggcttcatagaaaatggttgggagggaatgatggacggttggtacggtttcaggcatcaaaattctgagggcacagggcaagcagcagatcttaaaagcactcaagcagcaatcaaccaaatcaacgggaaactgaataggttaatcgagaaaacgaacgagaaattccatcaaattgaaaaagaattctcagaagtagaagggagaattcaggacctcgagaaatatgttgaggacactaaaatagatctctggtcgtacaatgcggagcttcttgttgccctggagaaccaacatacaattgatctaactgactcagaaatgaacaaactgtttgaaagaacaaagaagcaactgagggaaaatgctgaggatatgggcaatggttgtttcaaaatataccacaaatgtgacaatgcctgcatagggtcaatcagaaatggaacttatgaccatgatgtatacagagacgaagcattgaacaaccggttccagatcaaaggtgttgagctgaagtcaggatacaaagattggatcctatggatttcctttgccatatcatgttttttgctttgtattgttttgctggggttcatcatgtgggcctgccaaaaaggcaacattaggtgcaacatttgcatttga